European Patent Application EP 4 733 765 A2, published April 29, 2026. Title: Pulmonary hypertension improving composition, method for predicting prognosis of pulmonary hypertension, method for assisting determining severity of pulmonary hypertension, and method for assisting diagnosis of pulmonary hypertension. Applicant: Nakaoka, Yoshikazu. Application EP 25 226 931.1, filed February 21, 2020. The sequence listing filed with the application follows.

SEQUENCE LISTING (10 sequences)

SEQ ID NO: 1 - DNA, 20 bp, synthetic construct
  misc_feature 1..20: note = Primer
  source 1..20: mol_type = other DNA
gtgstgcayggytgtcgtca

SEQ ID NO: 2 - DNA, 20 bp, synthetic construct
  misc_feature 1..20: note = Primer
  source 1..20: mol_type = other DNA
acgtcrtccmcaccttcctc

SEQ ID NO: 3 - DNA, 20 bp, synthetic construct
  misc_feature 1..20: note = Primer
  source 1..20: mol_type = other DNA
gcctagcttgctaggtggat

SEQ ID NO: 4 - DNA, 20 bp, synthetic construct
  misc_feature 1..20: note = Primer
  source 1..20: mol_type = other DNA
gcaggtaccgtcaatctctc

SEQ ID NO: 5 - DNA, 23 bp, synthetic construct
  misc_feature 1..23: note = Primer
  source 1..23: mol_type = other DNA
gtacagttgcttcaggacgtatc

SEQ ID NO: 6 - DNA, 21 bp, synthetic construct
  misc_feature 1..21: note = Primer
  source 1..21: mol_type = other DNA
acgttcgatttcatcacgttg

SEQ ID NO: 7 - DNA, 22 bp, synthetic construct
  misc_feature 1..22: note = Primer
  source 1..22: mol_type = other DNA
gacggaaagaccccgtgaacct

SEQ ID NO: 8 - DNA, 20 bp, synthetic construct
  misc_feature 1..20: note = Primer
  source 1..20: mol_type = other DNA
ggcaagtttcgtgcttagat

SEQ ID NO: 9 - DNA, 20 bp, synthetic construct
  misc_feature 1..20: note = Primer
  source 1..20: mol_type = other DNA
agrgtttgatcmtggctcag

SEQ ID NO: 10 - DNA, 19 bp, synthetic construct
  misc_feature 1..19: note = Primer
  source 1..19: mol_type = other DNA
tgctgcctcccgtaggagt